European Patent Application EP 4 265 638 A1, published October 25, 2023. Title: CHIMERIC ANTIGEN RECEPTOR TARGETING CD123 AND USE THEREOF. Applicant: BEIJING IMMUNOCHINA PHARMACEUTICALS CO., LTD. SHANDONG JINSAI CO., LTD. The sequence listing filed with the application follows.

SEQUENCE LISTING (70 sequences)

SEQ ID NO: 1 - protein, 11 aa, Synthetic sequence
  The amino acid at position 3 is selected from Ser and Thr; the amino acid at position 4 is selected from Phe and Ile; the amino acid at position 5 is selected from Thr, Ser and Met; the amino acid at position 6 is selected from Ser, Asp, Thr, Gly; the amino acid position 9 is selected from Trp, Tyr, Val, Ala and Asn; the amino acid at position 10 is selected from Met, Val, Ile and Trp; and the amino acid at position 11 is selected from Asn and His;
GYXXXXDYXXX

SEQ ID NO: 2 - protein, 19 aa, Synthetic sequence
  The amino acid at position 1 is selected from Tyr and Arg; the amino acid at position 2 is selected from Ile and Cys; the amino acid at position 3 is selected from Asp, Asn, Tyr and Ser; the amino acid at position 4 is selected from Pro and Cys; the amino acid at position 5 is selected from Tyr and Gly; the amino acid at position 6 is selected from Asp, Asn and Ser; the amino acid at position 7 is selected from Ser, Asn, Asp and Gly; the amino acid at position 8 is selected from Glu, Ala, Gly and Ser; the amino acid at position 9 is selected from Thr, Ile and Ser; the amino acid at position 10 is selected from His, Ser and Asn; the amino acid at position 11 is selected from Tyr and Ser; the amino acid at position 13 is selected from Gln, Glu and Pro; the amino acid at position 14 is selected from Lys, Asn and Ser; the amino acid at position 15 is selected from Phe and Leu; the amino acid at position 17 is selected from Asp, Gly and Ser; the amino acid at position 18 is selected from Lys and Arg; and the amino acid at position 19 is selected from Ala and Ile;
XXXXXXXXXXXNXXXKXXX

SEQ ID NO: 3 - protein, 19 aa, Synthetic sequence
  the amino acid at position 2 is selected from Arg and Gly; the amino acid at position 3 is selected from Gly, Ser and Glu; the amino acid at position 4 is selected from Glu, Pro and Arg; the amino acid at position 5 is selected from Gly and Ser; the amino acid at position 6 is selected from Asn, Tyr, Leu and Trp; the amino acid at position 7 is selected from Trp, Tyr, Leu; the amino acid at position 8 is selected from Gly and Asp; the amino acid at position 11 is selected from Arg and Glu; the amino acid at position 12 is selected from Tyr, Ser and Thr; the amino acid at position 13 is selected from Asp, Tyr and Gly; the amino acid at position 14 is selected from Gly and Tyr; the amino acid at position 15 is selected from Tyr and Leu; the amino acid at position 16 is selected from Ala, Gly and Pro; the amino acid at position 17 is selected from Met and Leu; the amino acid at position 18 is selected from Asp and Ala; and the amino acid at position 19 is selected from Tyr and Cys;
AXXXXXXXYDXXXXXXXXX

SEQ ID NO: 4 - protein, 17 aa, Synthetic sequence
  the amino acid at position 1 is selected from Ala and Ser; the amino acid at position 3 is selected from Gln, Lys and Ser; the amino acid at position 4 is selected from Ser and Asp; the amino acid at position 5 is selected from Ile, Val, Leu; the amino acid at position 6 is selected from Ser, Asn, Asp and Leu; the amino acid at position 7 is selected from Lys, Tyr, Ser, Asp and Asn; the amino acid at position 8 is selected from Asp and Ser; the amino acid at position 9 is selected from Gly and Ser; the amino acid at position 10 is selected from Asp and Asn; the amino acid at position 13 is selected from Ser and Asn; the amino acid at position 14 is selected from Asp and Tyr; the amino acid at position 15 is selected from Leu, Ile and Met; and the amino acid at position 16 is selected from Ala, Asn and His;
XSXXXXXXXXQKXXXXW

SEQ ID NO: 5 - protein, 7 aa, Synthetic sequence
  the amino acid at position 1 is selected from Gly, Thr and Ala; the amino acid at position 3 is selected from Thr, Asn and Gln; the amino acid at position 4 is selected from Leu, Ser and Arg; the amino acid at position 5 is selected from Gln, Glu, Ala, Ile and Asp; the amino acid at position 6 is selected from Ser and Pro; and the amino acid at position 7 is selected from Gly and Glu;
XSXXXXX

SEQ ID NO: 6 - protein, 9 aa, Synthetic sequence
  the amino acid at position 1 is selected from Gln and Asn; the amino acid at position 2 is selected from His, Tyr, Ser, Phe and Gly; the amino acid at position 3 is selected from Asn, Asp, His and Tyr; the amino acid at position 4 is selected from Lys, Leu, Glu, Arg and Ser; the amino acid at position 5 is selected from Tyr, Leu, Asp, Ser, Phe and Thr; and the amino acid at position 7 is selected from Tyr, Arg and Trp;
XXXXXPXTF

SEQ ID NO: 7 - protein, 10 aa, Synthetic sequence
GYTFTSYWMN

SEQ ID NO: 8 - protein, 10 aa, Synthetic sequence
GYSFTDYYVH

SEQ ID NO: 9 - protein, 10 aa, Synthetic sequence
GYTFMTYVIH

SEQ ID NO: 10 - protein, 11 aa, Synthetic sequence
GYSITSDYAWN

SEQ ID NO: 11 - protein, 10 aa, Synthetic sequence
GYTFSSYNMH

SEQ ID NO: 12 - protein, 10 aa, Synthetic sequence
GYSFTGYYMH

SEQ ID NO: 13 - protein, 19 aa, Synthetic sequence
RIDPYDSETHYNQKFKDKA

SEQ ID NO: 14 - protein, 19 aa, Synthetic sequence
YISCYNGATNYNPKFKGKA

SEQ ID NO: 15 - protein, 19 aa, Synthetic sequence
YCNPYNDGINYNEKFKGKA

SEQ ID NO: 16 - protein, 18 aa, Synthetic sequence
YISYSGSSNSNPSLKSRI

SEQ ID NO: 17 - protein, 19 aa, Synthetic sequence
YIYPGNGGTNYNQKFKGKA

SEQ ID NO: 18 - protein, 19 aa, Synthetic sequence
RINPYNNATSYNQNFKDKA

SEQ ID NO: 19 - protein, 8 aa, Synthetic sequence
ARGNWDDY

SEQ ID NO: 20 - protein, 16 aa, Synthetic sequence
AGGEGYYGYDGYAMDY

SEQ ID NO: 21 - protein, 17 aa, Synthetic sequence
ARSPSYYGRSYYYGMDY

SEQ ID NO: 22 - protein, 6 aa, Synthetic sequence
ARGMDY

SEQ ID NO: 23 - protein, 19 aa, Synthetic sequence
ARERGLYDYDETGYYAMDY

SEQ ID NO: 24 - protein, 12 aa, Synthetic sequence
ARGEGWLLPLAC

SEQ ID NO: 25 - protein, 11 aa, Synthetic sequence
ASKSISKDLAW

SEQ ID NO: 26 - protein, 11 aa, Synthetic sequence
ASQDINKYIAW

SEQ ID NO: 27 - protein, 15 aa, Synthetic sequence
ASQSVDYDGDSYMNW

SEQ ID NO: 28 - protein, 12 aa, Synthetic sequence
ASSSVSSSYLHW

SEQ ID NO: 29 - protein, 11 aa, Synthetic sequence
ASQSISDYLHW

SEQ ID NO: 30 - protein, 17 aa, Synthetic sequence
SSQSLLNSSNQKNYLAW

SEQ ID NO: 31 - protein, 7 aa, Synthetic sequence
GSTLQSG

SEQ ID NO: 32 - protein, 7 aa, Synthetic sequence
TSTLQPG

SEQ ID NO: 33 - protein, 7 aa, Synthetic sequence
ASNLESG

SEQ ID NO: 34 - protein, 7 aa, Synthetic sequence
TSNLASG

SEQ ID NO: 35 - protein, 7 aa, Synthetic sequence
ASQSISE

SEQ ID NO: 36 - protein, 7 aa, Synthetic sequence
ASTRDSG

SEQ ID NO: 37 - protein, 9 aa, Synthetic sequence
QHNKYPYTF

SEQ ID NO: 38 - protein, 8 aa, Synthetic sequence
QYDDLYTF

SEQ ID NO: 39 - protein, 9 aa, Synthetic sequence
QSNEDPYTF

SEQ ID NO: 40 - protein, 9 aa, Synthetic sequence
QFHRSPRTF

SEQ ID NO: 41 - protein, 9 aa, Synthetic sequence
NGHSFPYTF

SEQ ID NO: 42 - protein, 9 aa, Synthetic sequence
QHYSTPWTF

SEQ ID NO: 43 - protein, 115 aa, Synthetic sequence
QVQLQQPGAELVRPGASVKLSCKASGYTFTSYWMNWVKQRPDQGLEWIGRIDPYDSETHYNQKFKDKAILTVDKSSSTAYMQLSSLTSEDSAVYYCARGNWDDYWGQGTTLTVSS

SEQ ID NO: 44 - protein, 123 aa, Synthetic sequence
QVQLKQSGPELVKTGASVKMSCKASGYSFTDYYVHWVRQSHGKSLEWIGYISCYNGATNYNPKFKGKATFTVDTSSSTAYMQFKSLTSEDSAVYYCAGGEGYYGYDGYAMDYWGQGTSVTVSS

SEQ ID NO: 45 - protein, 124 aa, Synthetic sequence
QVQLKQSGPELVKPGASVKMSCKASGYTFMTYVIHWVKQKPGQGLEWFGYCNPYNDGINYNEKFKGKATLTSDKSSSTVYMELSSLTSEDSAVYYCARSPSYYGRSYYYGMDYWGQGTSVTVSS

SEQ ID NO: 46 - protein, 113 aa, Synthetic sequence
DVKLQESGPGLVKPSQSLSLTCTVTGYSITSDYAWNWIRQFPGNKLEWMGYISYSGSSNSNPSLKSRISITRDTSKNQFFLQLNSVTTEDTATYYCARGMDYWGQGTSVTVSS

SEQ ID NO: 47 - protein, 126 aa, Synthetic sequence
QVQLKQSGAELVRSGASVKMSCKASGYTFSSYNMHWVKQTPGQGLEWIGYIYPGNGGTNYNQKFKGKATLTADTSSSTAYMQISSLTSEDSAVYFCARERGLYDYDETGYYAMDYWGQGTSVTVSS

SEQ ID NO: 48 - protein, 119 aa, Synthetic sequence
QVQLKQSGPELVKSGASVKISCKASGYSFTGYYMHWVKQSHVKSLEWIGRINPYNNATSYNQNFKDKASLTVDKSSSTAYMELHSLTSEDSAVYYCARGEGWLLPLACWGQGTLVTVSA

SEQ ID NO: 49 - protein, 107 aa, Synthetic sequence
DVQITQSPSYLAASPGETITINCRASKSISKDLAWYQEKPGKTNKLLIYSGSTLQSGIPSRFSGSGSGTDFTLTISSLEPEDFAMYYCQQHNKYPYTFGGGTKLEIK

SEQ ID NO: 50 - protein, 106 aa, Synthetic sequence
DIQLTQSPSSLSASLGGKVTITCKASQDINKYIAWYQHKPGKGPRLLIHYTSTLQPGIPSRFSGSGSGGDYSFSISNLEPEDIATYYCLQYDDLYTFGGGTKLEIK

SEQ ID NO: 51 - protein, 111 aa, Synthetic sequence
DIQLTQSPASLAVSLGQRATISCKASQSVDYDGDSYMNWYQQKPGQPPKVLIYAASNLESGIPARFSGSGSGTDFTLNIHPVEEEDAATYYCQQSNEDPYTFGGGTKLDIK

SEQ ID NO: 52 - protein, 108 aa, Synthetic sequence
DIVLTQSPAIMSVFLGERVTMTCTASSSVSSSYLHWYQQKPGSSPKLWIYSTSNLASGVPARFSGSGSGTSYSLTISSMEAEDAATYYCHQFHRSPRTFGGGTKLEIK

SEQ ID NO: 53 - protein, 107 aa, Synthetic sequence
DIQLTQSPATLSVTPGDRVSLSCRASQSISDYLHWYQQKSHESPRLLIKYASQSISEIPSRFSGSGSGSDFTLSINSVEPEDVGVYFCQNGHSFPYTFGGGTKLEIK

SEQ ID NO: 54 - protein, 113 aa, Synthetic sequence
DIVMTQSPSSLAMSVGQKVTMSCKSSQSLLNSSNQKNYLAWYQQKPGQSPKLLVYFASTRDSGVPDRFIGSGSGTDFTLTISSVQAEDLADYFCQQHYSTPWTFGGGTKLEIK

SEQ ID NO: 55 - protein, 237 aa, Synthetic sequence
QVQLQQPGAELVRPGASVKLSCKASGYTFTSYWMNWVKQRPDQGLEWIGRIDPYDSETHYNQKFKDKAILTVDKSSSTAYMQLSSLTSEDSAVYYCARGNWDDYWGQGTTLTVSSGGGGSGGGGSGGGGSDVQITQSPSYLAASPGETITINCRASKSISKDLAWYQEKPGKTNKLLIYSGSTLQSGIPSRFSGSGSGTDFTLTISSLEPEDFAMYYCQQHNKYPYTFGGGTKLEIK

SEQ ID NO: 56 - protein, 244 aa, Synthetic sequence
QVQLKQSGPELVKTGASVKMSCKASGYSFTDYYVHWVRQSHGKSLEWIGYISCYNGATNYNPKFKGKATFTVDTSSSTAYMQFKSLTSEDSAVYYCAGGEGYYGYDGYAMDYWGQGTSVTVSSGGGGSGGGGSGGGGSDIQLTQSPSSLSASLGGKVTITCKASQDINKYIAWYQHKPGKGPRLLIHYTSTLQPGIPSRFSGSGSGGDYSFSISNLEPEDIATYYCLQYDDLYTFGGGTKLEIK

SEQ ID NO: 57 - protein, 250 aa, Synthetic sequence
QVQLKQSGPELVKPGASVKMSCKASGYTFMTYVIHWVKQKPGQGLEWFGYCNPYNDGINYNEKFKGKATLTSDKSSSTVYMELSSLTSEDSAVYYCARSPSYYGRSYYYGMDYWGQGTSVTVSSGGGGSGGGGSGGGGSDIQLTQSPASLAVSLGQRATISCKASQSVDYDGDSYMNWYQQKPGQPPKVLIYAASNLESGIPARFSGSGSGTDFTLNIHPVEEEDAATYYCQQSNEDPYTFGGGTKLDIK

SEQ ID NO: 58 - protein, 236 aa, Synthetic sequence
DVKLQESGPGLVKPSQSLSLTCTVTGYSITSDYAWNWIRQFPGNKLEWMGYISYSGSSNSNPSLKSRISITRDTSKNQFFLQLNSVTTEDTATYYCARGMDYWGQGTSVTVSSGGGGSGGGGSGGGGSDIVLTQSPAIMSVFLGERVTMTCTASSSVSSSYLHWYQQKPGSSPKLWIYSTSNLASGVPARFSGSGSGTSYSLTISSMEAEDAATYYCHQFHRSPRTFGGGTKLEIK

SEQ ID NO: 59 - protein, 248 aa, Synthetic sequence
QVQLKQSGAELVRSGASVKMSCKASGYTFSSYNMHWVKQTPGQGLEWIGYIYPGNGGTNYNQKFKGKATLTADTSSSTAYMQISSLTSEDSAVYFCARERGLYDYDETGYYAMDYWGQGTSVTVSSGGGGSGGGGSGGGGSDIQLTQSPATLSVTPGDRVSLSCRASQSISDYLHWYQQKSHESPRLLIKYASQSISEIPSRFSGSGSGSDFTLSINSVEPEDVGVYFCQNGHSFPYTFGGGTKLEIK

SEQ ID NO: 60 - protein, 247 aa, Synthetic sequence
QVQLKQSGPELVKSGASVKISCKASGYSFTGYYMHWVKQSHVKSLEWIGRINPYNNATSYNQNFKDKASLTVDKSSSTAYMELHSLTSEDSAVYYCARGEGWLLPLACWGQGTLVTVSAGGGGSGGGGSGGGGSDIVMTQSPSSLAMSVGQKVTMSCKSSQSLLNSSNQKNYLAWYQQKPGQSPKLLVYFASTRDSGVPDRFIGSGSGTDFTLTISSVQAEDLADYFCQQHYSTPWTFGGGTKLEIK

SEQ ID NO: 61 - protein, 244 aa, Synthetic sequence
DIQLTQSPSSLSASLGGKVTITCKASQDINKYIAWYQHKPGKGPRLLIHYTSTLQPGIPSRFSGSGSGGDYSFSISNLEPEDIATYYCLQYDDLYTFGGGTKLEIKGGGGSGGGGSGGGGSQVQLKQSGPELVKTGASVKMSCKASGYSFTDYYVHWVRQSHGKSLEWIGYISCYNGATNYNPKFKGKATFTVDTSSSTAYMQFKSLTSEDSAVYYCAGGEGYYGYDGYAMDYWGQGTSVTVSS

SEQ ID NO: 62 - protein, 42 aa, Synthetic sequence
KRGRKKLLYIFKQPFMRPVQTTQEEDGCSCRFPEEEEGGCEL

SEQ ID NO: 63 - protein, 112 aa, Synthetic sequence
RVKFSRSADAPAYKQGQNQLYNELNLGRREEYDVLDKRRGRDPEMGGKPRRKNPQEGLYNELQKDKMAEAYSEIGMKGERRRGKGHDGLYQGLSTATKDTYDALHMQALPPR

SEQ ID NO: 64 - protein, 501 aa, Synthetic sequence
MLLLVTSLLLCELPHPAFLLIPNWSHPQFEKGGGGSGGGGSQVQLQQPGAELVRPGASVKLSCKASGYTFTSYWMNWVKQRPDQGLEWIGRIDPYDSETHYNQKFKDKAILTVDKSSSTAYMQLSSLTSEDSAVYYCARGNWDDYWGQGTTLTVSSGGGGSGGGGSGGGGSDVQITQSPSYLAASPGETITINCRASKSISKDLAWYQEKPGKTNKLLIYSGSTLQSGIPSRFSGSGSGTDFTLTISSLEPEDFAMYYCQQHNKYPYTFGGGTKLEIKTTTPAPRPPTPAPTIASQPLSLRPEACRPAAGGAVHTRGLDFACDIYIWAPLAGTCGVLLLSLVITLYCKRGRKKLLYIFKQPFMRPVQTTQEEDGCSCRFPEEEEGGCELRVKFSRSADAPAYKQGQNQLYNELNLGRREEYDVLDKRRGRDPEMGGKPRRKNPQEGLYNELQKDKMAEAYSEIGMKGERRRGKGHDGLYQGLSTATKDTYDALHMQALPPR

SEQ ID NO: 65 - protein, 508 aa, Synthetic sequence
MLLLVTSLLLCELPHPAFLLIPNWSHPQFEKGGGGSGGGGSQVQLKQSGPELVKTGASVKMSCKASGYSFTDYYVHWVRQSHGKSLEWIGYISCYNGATNYNPKFKGKATFTVDTSSSTAYMQFKSLTSEDSAVYYCAGGEGYYGYDGYAMDYWGQGTSVTVSSGGGGSGGGGSGGGGSDIQLTQSPSSLSASLGGKVTITCKASQDINKYIAWYQHKPGKGPRLLIHYTSTLQPGIPSRFSGSGSGGDYSFSISNLEPEDIATYYCLQYDDLYTFGGGTKLEIKTTTPAPRPPTPAPTIASQPLSLRPEACRPAAGGAVHTRGLDFACDIYIWAPLAGTCGVLLLSLVITLYCKRGRKKLLYIFKQPFMRPVQTTQEEDGCSCRFPEEEEGGCELRVKFSRSADAPAYKQGQNQLYNELNLGRREEYDVLDKRRGRDPEMGGKPRRKNPQEGLYNELQKDKMAEAYSEIGMKGERRRGKGHDGLYQGLSTATKDTYDALHMQALPPR

SEQ ID NO: 66 - protein, 514 aa, Synthetic sequence
MLLLVTSLLLCELPHPAFLLIPNWSHPQFEKGGGGSGGGGSQVQLKQSGPELVKPGASVKMSCKASGYTFMTYVIHWVKQKPGQGLEWFGYCNPYNDGINYNEKFKGKATLTSDKSSSTVYMELSSLTSEDSAVYYCARSPSYYGRSYYYGMDYWGQGTSVTVSSGGGGSGGGGSGGGGSDIQLTQSPASLAVSLGQRATISCKASQSVDYDGDSYMNWYQQKPGQPPKVLIYAASNLESGIPARFSGSGSGTDFTLNIHPVEEEDAATYYCQQSNEDPYTFGGGTKLDIKTTTPAPRPPTPAPTIASQPLSLRPEACRPAAGGAVHTRGLDFACDIYIWAPLAGTCGVLLLSLVITLYCKRGRKKLLYIFKQPFMRPVQTTQEEDGCSCRFPEEEEGGCELRVKFSRSADAPAYKQGQNQLYNELNLGRREEYDVLDKRRGRDPEMGGKPRRKNPQEGLYNELQKDKMAEAYSEIGMKGERRRGKGHDGLYQGLSTATKDTYDALHMQALPPR

SEQ ID NO: 67 - protein, 500 aa, Synthetic sequence
MLLLVTSLLLCELPHPAFLLIPNWSHPQFEKGGGGSGGGGSDVKLQESGPGLVKPSQSLSLTCTVTGYSITSDYAWNWIRQFPGNKLEWMGYISYSGSSNSNPSLKSRISITRDTSKNQFFLQLNSVTTEDTATYYCARGMDYWGQGTSVTVSSGGGGSGGGGSGGGGSDIVLTQSPAIMSVFLGERVTMTCTASSSVSSSYLHWYQQKPGSSPKLWIYSTSNLASGVPARFSGSGSGTSYSLTISSMEAEDAATYYCHQFHRSPRTFGGGTKLEIKTTTPAPRPPTPAPTIASQPLSLRPEACRPAAGGAVHTRGLDFACDIYIWAPLAGTCGVLLLSLVITLYCKRGRKKLLYIFKQPFMRPVQTTQEEDGCSCRFPEEEEGGCELRVKFSRSADAPAYKQGQNQLYNELNLGRREEYDVLDKRRGRDPEMGGKPRRKNPQEGLYNELQKDKMAEAYSEIGMKGERRRGKGHDGLYQGLSTATKDTYDALHMQALPPR

SEQ ID NO: 68 - protein, 512 aa, Synthetic sequence
MLLLVTSLLLCELPHPAFLLIPNWSHPQFEKGGGGSGGGGSQVQLKQSGAELVRSGASVKMSCKASGYTFSSYNMHWVKQTPGQGLEWIGYIYPGNGGTNYNQKFKGKATLTADTSSSTAYMQISSLTSEDSAVYFCARERGLYDYDETGYYAMDYWGQGTSVTVSSGGGGSGGGGSGGGGSDIQLTQSPATLSVTPGDRVSLSCRASQSISDYLHWYQQKSHESPRLLIKYASQSISEIPSRFSGSGSGSDFTLSINSVEPEDVGVYFCQNGHSFPYTFGGGTKLEIKTTTPAPRPPTPAPTIASQPLSLRPEACRPAAGGAVHTRGLDFACDIYIWAPLAGTCGVLLLSLVITLYCKRGRKKLLYIFKQPFMRPVQTTQEEDGCSCRFPEEEEGGCELRVKFSRSADAPAYKQGQNQLYNELNLGRREEYDVLDKRRGRDPEMGGKPRRKNPQEGLYNELQKDKMAEAYSEIGMKGERRRGKGHDGLYQGLSTATKDTYDALHMQALPPR

SEQ ID NO: 69 - protein, 511 aa, Synthetic sequence
MLLLVTSLLLCELPHPAFLLIPNWSHPQFEKGGGGSGGGGSQVQLKQSGPELVKSGASVKISCKASGYSFTGYYMHWVKQSHVKSLEWIGRINPYNNATSYNQNFKDKASLTVDKSSSTAYMELHSLTSEDSAVYYCARGEGWLLPLACWGQGTLVTVSAGGGGSGGGGSGGGGSDIVMTQSPSSLAMSVGQKVTMSCKSSQSLLNSSNQKNYLAWYQQKPGQSPKLLVYFASTRDSGVPDRFIGSGSGTDFTLTISSVQAEDLADYFCQQHYSTPWTFGGGTKLEIKTTTPAPRPPTPAPTIASQPLSLRPEACRPAAGGAVHTRGLDFACDIYIWAPLAGTCGVLLLSLVITLYCKRGRKKLLYIFKQPFMRPVQTTQEEDGCSCRFPEEEEGGCELRVKFSRSADAPAYKQGQNQLYNELNLGRREEYDVLDKRRGRDPEMGGKPRRKNPQEGLYNELQKDKMAEAYSEIGMKGERRRGKGHDGLYQGLSTATKDTYDALHMQALPPR

SEQ ID NO: 70 - protein, 508 aa, Synthetic sequence
MLLLVTSLLLCELPHPAFLLIPNWSHPQFEKGGGGSGGGGSDIQLTQSPSSLSASLGGKVTITCKASQDINKYIAWYQHKPGKGPRLLIHYTSTLQPGIPSRFSGSGSGGDYSFSISNLEPEDIATYYCLQYDDLYTFGGGTKLEIKGGGGSGGGGSGGGGSQVQLKQSGPELVKTGASVKMSCKASGYSFTDYYVHWVRQSHGKSLEWIGYISCYNGATNYNPKFKGKATFTVDTSSSTAYMQFKSLTSEDSAVYYCAGGEGYYGYDGYAMDYWGQGTSVTVSSTTTPAPRPPTPAPTIASQPLSLRPEACRPAAGGAVHTRGLDFACDIYIWAPLAGTCGVLLLSLVITLYCKRGRKKLLYIFKQPFMRPVQTTQEEDGCSCRFPEEEEGGCELRVKFSRSADAPAYKQGQNQLYNELNLGRREEYDVLDKRRGRDPEMGGKPRRKNPQEGLYNELQKDKMAEAYSEIGMKGERRRGKGHDGLYQGLSTATKDTYDALHMQALPPR